European Patent Specification EP 3 664 776 B1, published May 14, 2025. Title: APTAMERS FOR CONSUMER PRODUCT COMPOSITIONS. Applicant: The Procter & Gamble Company Velasquez, Juan E. Trejo, Amy V. Sagel, Paul A. Penner, Gregoroy A. The sequence listing filed with the application follows.

SEQUENCE LISTING (222 sequences)

SEQ ID NO: 1 - RNA, 82 nt, Artificial Sequence
  Synthetic aptamer sequence
gggaagagaaggacauaugauucaugugagaugauguguguuccuaguuuuaucuugcucuuugacuaguacaugaccacuu

SEQ ID NO: 2 - RNA, 82 nt, Artificial Sequence
  Synthetic aptamer sequence
gggaagagaaggacauaugauuaggcuaacuguucagggauuugauaugcaugaggagcacuugacuaguacaugaccacuu

SEQ ID NO: 3 - RNA, 82 nt, Artificial Sequence
  Synthetic aptamer sequence
gggaagagaaggacauaugauccgcucuaaaguaccaaccgcgggagcuaaaugcaagccguugacuaguacaugaccacuu

SEQ ID NO: 4 - RNA, 82 nt, Artificial Sequence
  Synthetic aptamer sequence
gggaagagaaggacauaugauugugucaggcucuagagucuagacggccggggucccggauuugacuaguacaugaccacuu

SEQ ID NO: 5 - RNA, 82 nt, Artificial Sequence
  Synthetic aptamer sequence
gggaagagaaggacauaugauccuuaugucuagcggccuuacgcgauuaguggcguuuuguuugacuaguacaugaccacuu

SEQ ID NO: 6 - RNA, 82 nt, Artificial Sequence
  Synthetic aptamer sequence
gggaagagaaggacauaugaucuuuauguauuaucagucauaccggacgcagcccgcuggauugacuaguacaugaccacuu

SEQ ID NO: 7 - RNA, 82 nt, Artificial Sequence
  Synthetic aptamer sequence
gggaagagaaggacauaugauuguguuauuacacuucgugauuuuccuugcuuuucuauuuuugacuaguacaugaccacuu

SEQ ID NO: 8 - RNA, 82 nt, Artificial Sequence
  Synthetic aptamer sequence
gggaagagaaggacauaugauccaacaucuaaaguacuggucgccuagggagacuguucgguugacuaguacaugaccacuu

SEQ ID NO: 9 - RNA, 82 nt, Artificial Sequence
  Synthetic aptamer sequence
gggaagagaaggacauaugaugcuauauucgcaaaagcaggcugagugcggcaggcgcguguugacuaguacaugaccacuu

SEQ ID NO: 10 - RNA, 82 nt, Artificial Sequence
  Synthetic aptamer sequence
gggaagagaaggacauaugauucauucauucgcaacacaauuguauucgcaucugcgauuuuugacuaguacaugaccacuu

SEQ ID NO: 11 - RNA, 82 nt, Artificial Sequence
  Synthetic aptamer sequence
gggaagagaaggacauaugaucuuucucuuuucuaauauuuaauuuauuggguaccaauuuuugacuaguacaugaccacuu

SEQ ID NO: 12 - RNA, 82 nt, Artificial Sequence
  Synthetic aptamer sequence
gggaagagaaggacauaugaucuuuguuucgcauacguuuucuuuuucucucuucuuauuuuugacuaguacaugaccacuu

SEQ ID NO: 13 - RNA, 82 nt, Artificial Sequence
  Synthetic aptamer sequence
gggaagagaaggacauaugauuauucuguucuucaaaaaucuuuuagcguauacgcuauuuuugacuaguacaugaccacuu

SEQ ID NO: 14 - RNA, 82 nt, Artificial Sequence
  Synthetic aptamer sequence
gggaagagaaggacauaugauuuccuuauguucggucaacagggacugcugcagcaccggcuugacuaguacaugaccacuu

SEQ ID NO: 15 - RNA, 82 nt, Artificial Sequence
  Synthetic aptamer sequence
gggaagagaaggacauaugauuaagcgcacucaacagggucuaugauccgcgccgaucauguugacuaguacaugaccacuu

SEQ ID NO: 16 - RNA, 82 nt, Artificial Sequence
  Synthetic aptamer sequence
gggaagagaaggacauaugauccgcuuuccauugagauuauaagcuguuagagacuuauuuuugacuaguacaugaccacuu

SEQ ID NO: 17 - RNA, 82 nt, Artificial Sequence
  Synthetic aptamer sequence
gggaagagaaggacauaugauuuucgaaacguuucuuucaaguucuuaaucauucccauuuuugacuaguacaugaccacuu

SEQ ID NO: 18 - RNA, 82 nt, Artificial Sequence
  Synthetic aptamer sequence
gggaagagaaggacauaugaucauuagaugcgcaguucgaagccgguacagcuggcgcgcguugacuaguacaugaccacuu

SEQ ID NO: 19 - RNA, 82 nt, Artificial Sequence
  Synthetic aptamer sequence
gggaagagaaggacauaugauaaagaauaaccuuaaaauaacaccaccgccucacagcauauugacuaguacaugaccacuu

SEQ ID NO: 20 - RNA, 82 nt, Artificial Sequence
  Synthetic aptamer sequence
gggaagagaaggacauaugauaaauugaucuauucuuuucggugcuauuuaucuuccauuuuugacuaguacaugaccacuu

SEQ ID NO: 21 - RNA, 82 nt, Artificial Sequence
  Synthetic aptamer sequence
gggaagagaaggacauaugaucuacucgcgcggcggacaaaagcgcaacccagcacccauguugacuaguacaugaccacuu

SEQ ID NO: 22 - RNA, 82 nt, Artificial Sequence
  Synthetic aptamer sequence
gggaagagaaggacauaugauucuuaguuuguaauuacuuuuccuuccuuuuauucuauuuuugacuaguacaugaccacuu

SEQ ID NO: 23 - RNA, 82 nt, Artificial Sequence
  Synthetic aptamer sequence
gggaagagaaggacauaugauaacccgcgcagacuuacaagcgcgcaaaaaaaggguacguuugacuaguacaugaccacuu

SEQ ID NO: 24 - RNA, 82 nt, Artificial Sequence
  Synthetic aptamer sequence
gggaagagaaggacauaugauauuccuuuaugccgcaucauuuuauuguuuaugacaauuuuugacuaguacaugaccacuu

SEQ ID NO: 25 - RNA, 82 nt, Artificial Sequence
  Synthetic aptamer sequence
gggaagagaaggacauaugauauuucguacuacuuuucuuccaagcuucaaucgcccauuuuugacuaguacaugaccacuu

SEQ ID NO: 26 - RNA, 82 nt, Artificial Sequence
  Synthetic aptamer sequence
gggaagagaaggacauaugauucacucauucgcaacacaauuguauucgcaucugcgauuuuugacuaguacaugaccacuu

SEQ ID NO: 27 - RNA, 82 nt, Artificial Sequence
  Synthetic aptamer sequence
gggaagagaaggacauaugauauuauuuccacaguuccuuuauccacacaucuucucauuuuugacuaguacaugaccacuu

SEQ ID NO: 28 - RNA, 82 nt, Artificial Sequence
  Synthetic aptamer sequence
gggaagagaaggacauaugauaaacucguuaucuauucguuuauuugcaucucuuucauuuuugacuaguacaugaccacuu

SEQ ID NO: 29 - RNA, 82 nt, Artificial Sequence
  Synthetic aptamer sequence
gggaagagaaggacauaugauccaaccucuaaaguacuggucgccuagggagacuguucgguugacuaguacaugaccacuu

SEQ ID NO: 30 - RNA, 82 nt, Artificial Sequence
  Synthetic aptamer sequence
gggaagagaaggacauaugauuuccuuuuugcuauuuccguuaauguaaacucuccuauuuuugacuaguacaugaccacuu

SEQ ID NO: 31 - RNA, 82 nt, Artificial Sequence
  Synthetic aptamer sequence
gggaagagaaggacauaugauccuuauggccuaguagggauccgggcgccgaccagcgcgauugacuaguacaugaccacuu

SEQ ID NO: 32 - RNA, 82 nt, Artificial Sequence
  Synthetic aptamer sequence
gggaagagaaggacauaugaucgucugucuucuucgaauacguuuugggcuaagcccauuuuugacuaguacaugaccacuu

SEQ ID NO: 33 - RNA, 82 nt, Artificial Sequence
  Synthetic aptamer sequence
gggaagagaaggacauaugauucaaccaaacugccgacgaccgagguauguccuuauguacuugacuaguacaugaccacuu

SEQ ID NO: 34 - RNA, 82 nt, Artificial Sequence
  Synthetic aptamer sequence
gggaagagaaggacauaugauuacgggucugagcaaaagcgaaggaagcaggcgcagggauuugacuaguacaugaccacuu

SEQ ID NO: 35 - RNA, 82 nt, Artificial Sequence
  Synthetic aptamer sequence
gggaagagaaggacauaugauucucucauucgcaacacaauuguauucgcaucugcgauuuuugacuaguacaugaccacuu

SEQ ID NO: 36 - RNA, 82 nt, Artificial Sequence
  Synthetic aptamer sequence
gggaagagaaggacauaugaugcucuaaaguacuaagcguuugcgccgaugcccggaccgcuugacuaguacaugaccacuu

SEQ ID NO: 37 - RNA, 82 nt, Artificial Sequence
  Synthetic aptamer sequence
gggaagagaaggacauaugauacuucauuaaugugaggccgucagggggcaaccuucgagcuugacuaguacaugaccacuu

SEQ ID NO: 38 - RNA, 82 nt, Artificial Sequence
  Synthetic aptamer sequence
gggaagagaaggacauaugauuccuuauucuuguuacuacuuucuuuuccuauuuuuuucuuugacuaguacaugaccacuu

SEQ ID NO: 39 - RNA, 82 nt, Artificial Sequence
  Synthetic aptamer sequence
gggaagagaaggacauaugaucguuauuuucauuuucuuguuccccauaugcccaggcgcauugacuaguacaugaccacuu

SEQ ID NO: 40 - RNA, 82 nt, Artificial Sequence
  Synthetic aptamer sequence
gggaagagaaggacauaugauaccagcggcguagaaacguacagcucgccuguaacgccuguugacuaguacaugaccacuu

SEQ ID NO: 41 - RNA, 82 nt, Artificial Sequence
  Synthetic aptamer sequence
gggaagagaaggacauaugaucgauaugggugcgggaauguacguucaccgaauaugcuccuugacuaguacaugaccacuu

SEQ ID NO: 42 - RNA, 82 nt, Artificial Sequence
  Synthetic aptamer sequence
gggaagagaaggacauaugauuaacagugcguagucauaucgaauguuuaucuuccuauuuuugacuaguacaugaccacuu

SEQ ID NO: 43 - RNA, 82 nt, Artificial Sequence
  Synthetic aptamer sequence
gggaagagaaggacauaugaucagacucucgcccaauucgcaaggcguugcauugcgauuuuugacuaguacaugaccacuu

SEQ ID NO: 44 - RNA, 82 nt, Artificial Sequence
  Synthetic aptamer sequence
gggaagagaaggacauaugauuuccaacucuccacgagagcaugggucgaaugacucauuuuugacuaguacaugaccacuu

SEQ ID NO: 45 - RNA, 82 nt, Artificial Sequence
  Synthetic aptamer sequence
gggaagagaaggacauaugaugcaucgcgcgucacucaacucgugauuaccgagggcgccguugacuaguacaugaccacuu

SEQ ID NO: 46 - RNA, 82 nt, Artificial Sequence
  Synthetic aptamer sequence
gggaagagaaggacauaugaucugaaucuuuccgcagcccuguccuuuuaaagacagguuuuugacuaguacaugaccacuu

SEQ ID NO: 47 - RNA, 82 nt, Artificial Sequence
  Synthetic aptamer sequence
gggaagagaaggacauaugauuuuguuacuuacuucgucuaucuucuguugcacacaguuuuugacuaguacaugaccacuu

SEQ ID NO: 48 - RNA, 82 nt, Artificial Sequence
  Synthetic aptamer sequence
gggaagagaaggacauaugauucaaaucuucagcgauaauggcacaauuuccgcgccauuuuugacuaguacaugaccacuu

SEQ ID NO: 49 - RNA, 82 nt, Artificial Sequence
  Synthetic aptamer sequence
gggaagagaaggacauaugauuuaugugagaugauguguguuccuaguuuuaucuugcucuuugacuaguacaugaccacuu

SEQ ID NO: 50 - RNA, 82 nt, Artificial Sequence
  Synthetic aptamer sequence
gggaagagaaggacauaugauccacuuuuccauuaacuguugcgggcaaguagcaccguuuuugacuaguacaugaccacuu

SEQ ID NO: 51 - RNA, 82 nt, Artificial Sequence
  Synthetic aptamer sequence
gggaagagaaggacauaugauagagaagaccauucggaaagagcugcguguccuuauguacuugacuaguacaugaccacuu

SEQ ID NO: 52 - RNA, 82 nt, Artificial Sequence
  Synthetic aptamer sequence
gggaagagaaggacauaugauucuuauguagcaagcaaaaugugccgccgagccgacgccauugacuaguacaugaccacuu

SEQ ID NO: 53 - RNA, 82 nt, Artificial Sequence
  Synthetic aptamer sequence
gggaagagaaggacauaugauaagcgcauaauaagccagccaguucuuggcgcgcgggguauugacuaguacaugaccacuu

SEQ ID NO: 54 - RNA, 82 nt, Artificial Sequence
  Synthetic aptamer sequence
gggaagagaaggacauaugauuaguccgcauuucuauuuucuauauggcuuacugccauuuuugacuaguacaugaccacuu

SEQ ID NO: 55 - RNA, 82 nt, Artificial Sequence
  Synthetic aptamer sequence
gggaagagaaggacauaugauauaaagaacacgcaaaaccacccggacacccggugccguguugacuaguacaugaccacuu

SEQ ID NO: 56 - RNA, 82 nt, Artificial Sequence
  Synthetic aptamer sequence
gggaagagaaggacauaugauacacaggcgguggagccgaagggcaccgggacaaaccgacuugacuaguacaugaccacuu

SEQ ID NO: 57 - RNA, 82 nt, Artificial Sequence
  Synthetic aptamer sequence
gggaagagaaggacauaugauaguuccggcgcagcagcguccucacguuuuacgugccccauugacuaguacaugaccacuu

SEQ ID NO: 58 - RNA, 82 nt, Artificial Sequence
  Synthetic aptamer sequence
gggaagagaaggacauaugaugaccgucgcgaucguuuauaauguucuggaucuuucauuuuugacuaguacaugaccacuu

SEQ ID NO: 59 - RNA, 82 nt, Artificial Sequence
  Synthetic aptamer sequence
gggaagagaaggacauaugauaaguggggccccgacgacuuuuccuuccucucuuccggcauugacuaguacaugaccacuu

SEQ ID NO: 60 - RNA, 82 nt, Artificial Sequence
  Synthetic aptamer sequence
gggaagagaaggacauaugauaucaacauaccaaaaugucauuuccaaucuuuucccauuuuugacuaguacaugaccacuu

SEQ ID NO: 61 - RNA, 82 nt, Artificial Sequence
  Synthetic aptamer sequence
gggaagagaaggacauaugauagcgaacaaacaagggugcccaggcccccuucgcacaucguugacuaguacaugaccacuu

SEQ ID NO: 62 - RNA, 82 nt, Artificial Sequence
  Synthetic aptamer sequence
gggaagagaaggacauaugauccucuguaacgcaaagucaagucgcgcaaggccgcccgcguugacuaguacaugaccacuu

SEQ ID NO: 63 - RNA, 82 nt, Artificial Sequence
  Synthetic aptamer sequence
gggaagagaaggacauaugaucuucaucugcgauuacgguacacuuuaguguaucguuuuuuugacuaguacaugaccacuu

SEQ ID NO: 64 - RNA, 82 nt, Artificial Sequence
  Synthetic aptamer sequence
gggaagagaaggacauaugaugccuaugugcuagaugcagcagcaaccgccggcgacuggauugacuaguacaugaccacuu

SEQ ID NO: 65 - RNA, 82 nt, Artificial Sequence
  Synthetic aptamer sequence
gggaagagaaggacauaugauccgcgcccuaaccuucugaccaagcuucccuggcacuugguugacuaguacaugaccacuu

SEQ ID NO: 66 - RNA, 82 nt, Artificial Sequence
  Synthetic aptamer sequence
gggaagagaaggacauaugauccuuauguauuaucagucauaccggacgcagcccgcuggauugacuaguacaugaccacuu

SEQ ID NO: 67 - RNA, 82 nt, Artificial Sequence
  Synthetic aptamer sequence
gggaagagaaggacauaugaucuaaucuauacuggcugcuaacgcuuuuucuuuuccauuuuugacuaguacaugaccacuu

SEQ ID NO: 68 - RNA, 82 nt, Artificial Sequence
  Synthetic aptamer sequence
gggaagagaaggacauaugaucaguuuacgcggagucguuuguguccauuucuucucauuuuugacuaguacaugaccacuu

SEQ ID NO: 69 - RNA, 82 nt, Artificial Sequence
  Synthetic aptamer sequence
gggaagagaaggacauaugauucacgugagaugauguguguuccuaguuuuaucuugcucuuugacuaguacaugaccacuu

SEQ ID NO: 70 - RNA, 82 nt, Artificial Sequence
  Synthetic aptamer sequence
gggaagagaaggacauaugauuccuuguguaccgcuccgaaugugcuccagcgcgccucgguugacuaguacaugaccacuu

SEQ ID NO: 71 - RNA, 82 nt, Artificial Sequence
  Synthetic aptamer sequence
gggaagagaaggacauaugauaagccggcccgggaacaugucacgcgcgcgcgcaaaguaguugacuaguacaugaccacuu

SEQ ID NO: 72 - RNA, 82 nt, Artificial Sequence
  Synthetic aptamer sequence
gggaagagaaggacauaugauccuggauuuccgaaauuagagugccguuucguuacgguuuuugacuaguacaugaccacuu

SEQ ID NO: 73 - RNA, 82 nt, Artificial Sequence
  Synthetic aptamer sequence
gggaagagaaggacauaugaucgugucauccgcacaaggaggccugcauggcagggacacguugacuaguacaugaccacuu

SEQ ID NO: 74 - RNA, 82 nt, Artificial Sequence
  Synthetic aptamer sequence
gggaagagaaggacauaugaugaguagacuuuuuguaucauuuuuuuaucguaagauauuuuugacuaguacaugaccacuu

SEQ ID NO: 75 - RNA, 82 nt, Artificial Sequence
  Synthetic aptamer sequence
gggaagagaaggacauaugauccaugugagaugauguguguuccuaguuuuaucuugcucuuugacuaguacaugaccacuu

SEQ ID NO: 76 - RNA, 82 nt, Artificial Sequence
  Synthetic aptamer sequence
gggaagagaaggacauaugaucuuugcucuagaguguagucuaugagggacaagguagccauugacuaguacaugaccacuu

SEQ ID NO: 77 - RNA, 82 nt, Artificial Sequence
  Synthetic aptamer sequence
gggaagagaaggacauaugauguugguuuucuuucucuuucuuuucuuucucuuucuauuuuugacuaguacaugaccacuu

SEQ ID NO: 78 - RNA, 82 nt, Artificial Sequence
  Synthetic aptamer sequence
gggaagagaaggacauaugaucaaucgggcggggguaagaggcgugcgcagcguggagguguugacuaguacaugaccacuu

SEQ ID NO: 79 - RNA, 82 nt, Artificial Sequence
  Synthetic aptamer sequence
gggaagagaaggacauaugaucaccguggugcgcaaagccgcaacgagaacugcggaaucguugacuaguacaugaccacuu

SEQ ID NO: 80 - RNA, 82 nt, Artificial Sequence
  Synthetic aptamer sequence
gggaagagaaggacauaugauugcuuuaagucuuuuuaucauuuuguuuccuucauuuuuuuugacuaguacaugaccacuu

SEQ ID NO: 81 - RNA, 82 nt, Artificial Sequence
  Synthetic aptamer sequence
gggaagagaaggacauaugaucgacuaguuauacugcaaaggcuauaagcgcgagcgcgcguugacuaguacaugaccacuu

SEQ ID NO: 82 - RNA, 82 nt, Artificial Sequence
  Synthetic aptamer sequence
gggaagagaaggacauaugaugaguaauagauggcguacacaaaucggauacgacgagcgcuugacuaguacaugaccacuu

SEQ ID NO: 83 - RNA, 82 nt, Artificial Sequence
  Synthetic aptamer sequence
gggaagagaaggacauaugauuuucgcuucaagauucccaacgccuuguaagucaagguuuuugacuaguacaugaccacuu

SEQ ID NO: 84 - RNA, 82 nt, Artificial Sequence
  Synthetic aptamer sequence
gggaagagaaggacauaugaugugugagaugagccccuggaccagacgcacgcucgcacuguugacuaguacaugaccacuu

SEQ ID NO: 85 - RNA, 82 nt, Artificial Sequence
  Synthetic aptamer sequence
gggaagagaaggacauaugaucaggaugcggcgccgguaauugacuucccccuacguaggauugacuaguacaugaccacuu

SEQ ID NO: 86 - RNA, 82 nt, Artificial Sequence
  Synthetic aptamer sequence
gggaagagaaggacauaugaucagggacccggccggugcaucuccuucuuuagcguacgccuugacuaguacaugaccacuu

SEQ ID NO: 87 - RNA, 82 nt, Artificial Sequence
  Synthetic aptamer sequence
gggaagagaaggacauaugaucugcucuaaaguaccaaccgcgggagcuaaaugcaagccguugacuaguacaugaccacuu

SEQ ID NO: 88 - RNA, 82 nt, Artificial Sequence
  Synthetic aptamer sequence
gggaagagaaggacauaugaugauugccaugcauuagggggggacgcgcgcgaaagggagauugacuaguacaugaccacuu

SEQ ID NO: 89 - RNA, 82 nt, Artificial Sequence
  Synthetic aptamer sequence
gggaagagaaggacauaugauucgcucuaaaguaccaaccgcgggagcuaaaugcaagccguugacuaguacaugaccacuu

SEQ ID NO: 90 - RNA, 82 nt, Artificial Sequence
  Synthetic aptamer sequence
gggaagagaaggacauaugauaaaaaaccgggguucuuaauuuucauuguucgucguacuuuugacuaguacaugaccacuu

SEQ ID NO: 91 - RNA, 82 nt, Artificial Sequence
  Synthetic aptamer sequence
gggaagagaaggacauaugauaacccauuggugaaucgcaaccacagccagcccggcgcgauugacuaguacaugaccacuu

SEQ ID NO: 92 - RNA, 82 nt, Artificial Sequence
  Synthetic aptamer sequence
gggaagagaaggacauaugaucgaagugaggggaucgcgcggggugcaccuaaauaugggauugacuaguacaugaccacuu

SEQ ID NO: 93 - RNA, 82 nt, Artificial Sequence
  Synthetic aptamer sequence
gggaagagaaggacauaugauagccuuauguacuauagaagucagcuauccgccgcacaauuugacuaguacaugaccacuu

SEQ ID NO: 94 - RNA, 82 nt, Artificial Sequence
  Synthetic aptamer sequence
gggaagagaaggacauaugaucguuguuuuucccaaagcucguuagcauucauuccuauuuuugacuaguacaugaccacuu

SEQ ID NO: 95 - RNA, 82 nt, Artificial Sequence
  Synthetic aptamer sequence
gggaagagaaggacauaugaugaucaucagcggaaagcacgaaacgccacgggccgcggcauugacuaguacaugaccacuu

SEQ ID NO: 96 - RNA, 82 nt, Artificial Sequence
  Synthetic aptamer sequence
gggaagagaaggacauaugauuccuuccuauugacaaugcgcccgggccucuucaauuguauugacuaguacaugaccacuu

SEQ ID NO: 97 - RNA, 82 nt, Artificial Sequence
  Synthetic aptamer sequence
gggaagagaaggacauaugauaguugccgcgcggcgcaagauuggagagucccgggcuguauugacuaguacaugaccacuu

SEQ ID NO: 98 - RNA, 82 nt, Artificial Sequence
  Synthetic aptamer sequence
gggaagagaaggacauaugaucauaaguucguucauuccguuaacacgcguauggcguuuuuugacuaguacaugaccacuu

SEQ ID NO: 99 - RNA, 82 nt, Artificial Sequence
  Synthetic aptamer sequence
gggaagagaaggacauaugauccuuugucuccaaaucuuaggacugaaugagugccuauuuuugacuaguacaugaccacuu

SEQ ID NO: 100 - RNA, 82 nt, Artificial Sequence
  Synthetic aptamer sequence
gggaagagaaggacauaugaucuucuuugagaauucucuuuuuacaauuccggcgccgugauugacuaguacaugaccacuu

SEQ ID NO: 101 - RNA, 82 nt, Artificial Sequence
  Synthetic aptamer sequence
gggaagagaaggacauaugauuaggcuaacuguuuagggauuugauaugcaugaggagcacuugacuaguacaugaccacuu

SEQ ID NO: 102 - RNA, 82 nt, Artificial Sequence
  Synthetic aptamer sequence
gggaagagaaggacauaugauuaggcuaacuguucagggaguugauaugcaugaggagcacuugacuaguacaugaccacuu

SEQ ID NO: 103 - RNA, 82 nt, Artificial Sequence
  Synthetic aptamer sequence
gggaagagaaggacauaugauuaggcuaacugcucagggauuugauaugcaugaggagcacuugacuaguacaugaccacuu

SEQ ID NO: 104 - RNA, 82 nt, Artificial Sequence
  Synthetic aptamer sequence
gggaagagaaggacauaugauuaggcuaacuguucagggacuugauaugcaugaggagcacuugacuaguacaugaccacuu

SEQ ID NO: 105 - RNA, 82 nt, Artificial Sequence
  Synthetic aptamer sequence
gggaagagaaggacauaugauuaggcucacuguucagggauuugauaugcaugaggagcacuugacuaguacaugaccacuu

SEQ ID NO: 106 - RNA, 82 nt, Artificial Sequence
  Synthetic aptamer sequence
gggaagagaaggacauaugauuaggcuaacuguucagggauuugauaugcauggggagcacuugacuaguacaugaccacuu

SEQ ID NO: 107 - RNA, 82 nt, Artificial Sequence
  Synthetic aptamer sequence
gggaagagaaggacauaugauuucuuccuauugacgaugcgcccgggccucuucaauuguauugacuaguacaugaccacuu

SEQ ID NO: 108 - RNA, 82 nt, Artificial Sequence
  Synthetic aptamer sequence
gggaagagaaggacauaugauuaggcuaacuguucggggauuugauaugcaugaggagcacuugacuaguacaugaccacuu

SEQ ID NO: 109 - RNA, 82 nt, Artificial Sequence
  Synthetic aptamer sequence
gggaagagaaggacauaugauuaggcuaacuguucagggauuugauaugcacgaggagcacuugacuaguacaugaccacuu

SEQ ID NO: 110 - RNA, 82 nt, Artificial Sequence
  Synthetic aptamer sequence
gggaagagaaggacauaugauuagguuaacuguucagggauuugauaugcaugaggagcacuugacuaguacaugaccacuu

SEQ ID NO: 111 - RNA, 82 nt, Artificial Sequence
  Synthetic aptamer sequence
gggaagagaaggacauaugauuaggcuaacuguucagggauuugaugugcaugaggagcacuugacuaguacaugaccacuu

SEQ ID NO: 112 - DNA, 82 bp, Artificial Sequence
  Synthetic aptamer sequence
gggaagagaaggacatatgattcatgtgagatgatgtgtgttcctagttttatcttgctctttgactagtacatgaccactt

SEQ ID NO: 113 - DNA, 82 bp, Artificial Sequence
  Synthetic aptamer sequence
gggaagagaaggacatatgattaggctaactgttcagggatttgatatgcatgaggagcacttgactagtacatgaccactt

SEQ ID NO: 114 - DNA, 82 bp, Artificial Sequence
  Synthetic aptamer sequence
gggaagagaaggacatatgatccgctctaaagtaccaaccgcgggagctaaatgcaagccgttgactagtacatgaccactt

SEQ ID NO: 115 - DNA, 82 bp, Artificial Sequence
  Synthetic aptamer sequence
gggaagagaaggacatatgattgtgtcaggctctagagtctagacggccggggtcccggatttgactagtacatgaccactt

SEQ ID NO: 116 - DNA, 82 bp, Artificial Sequence
  Synthetic aptamer sequence
gggaagagaaggacatatgatccttatgtctagcggccttacgcgattagtggcgttttgtttgactagtacatgaccactt

SEQ ID NO: 117 - DNA, 82 bp, Artificial Sequence
  Synthetic aptamer sequence
gggaagagaaggacatatgatctttatgtattatcagtcataccggacgcagcccgctggattgactagtacatgaccactt

SEQ ID NO: 118 - DNA, 82 bp, Artificial Sequence
  Synthetic aptamer sequence
gggaagagaaggacatatgattgtgttattacacttcgtgattttccttgcttttctatttttgactagtacatgaccactt

SEQ ID NO: 119 - DNA, 82 bp, Artificial Sequence
  Synthetic aptamer sequence
gggaagagaaggacatatgatccaacatctaaagtactggtcgcctagggagactgttcggttgactagtacatgaccactt

SEQ ID NO: 120 - DNA, 82 bp, Artificial Sequence
  Synthetic aptamer sequence
gggaagagaaggacatatgatgctatattcgcaaaagcaggctgagtgcggcaggcgcgtgttgactagtacatgaccactt

SEQ ID NO: 121 - DNA, 82 bp, Artificial Sequence
  Synthetic aptamer sequence
gggaagagaaggacatatgattcattcattcgcaacacaattgtattcgcatctgcgatttttgactagtacatgaccactt

SEQ ID NO: 122 - DNA, 82 bp, Artificial Sequence
  Synthetic aptamer sequence
gggaagagaaggacatatgatctttctcttttctaatatttaatttattgggtaccaatttttgactagtacatgaccactt

SEQ ID NO: 123 - DNA, 82 bp, Artificial Sequence
  Synthetic aptamer sequence
gggaagagaaggacatatgatctttgtttcgcatacgttttctttttctctcttcttatttttgactagtacatgaccactt

SEQ ID NO: 124 - DNA, 82 bp, Artificial Sequence
  Synthetic aptamer sequence
gggaagagaaggacatatgattattctgttcttcaaaaatcttttagcgtatacgctatttttgactagtacatgaccactt

SEQ ID NO: 125 - DNA, 82 bp, Artificial Sequence
  Synthetic aptamer sequence
gggaagagaaggacatatgatttccttatgttcggtcaacagggactgctgcagcaccggcttgactagtacatgaccactt

SEQ ID NO: 126 - DNA, 82 bp, Artificial Sequence
  Synthetic aptamer sequence
gggaagagaaggacatatgattaagcgcactcaacagggtctatgatccgcgccgatcatgttgactagtacatgaccactt

SEQ ID NO: 127 - DNA, 82 bp, Artificial Sequence
  Synthetic aptamer sequence
gggaagagaaggacatatgatccgctttccattgagattataagctgttagagacttatttttgactagtacatgaccactt

SEQ ID NO: 128 - DNA, 82 bp, Artificial Sequence
  Synthetic aptamer sequence
gggaagagaaggacatatgattttcgaaacgtttctttcaagttcttaatcattcccatttttgactagtacatgaccactt

SEQ ID NO: 129 - DNA, 82 bp, Artificial Sequence
  Synthetic aptamer sequence
gggaagagaaggacatatgatcattagatgcgcagttcgaagccggtacagctggcgcgcgttgactagtacatgaccactt

SEQ ID NO: 130 - DNA, 82 bp, Artificial Sequence
  Synthetic aptamer sequence
gggaagagaaggacatatgataaagaataaccttaaaataacaccaccgcctcacagcatattgactagtacatgaccactt

SEQ ID NO: 131 - DNA, 82 bp, Artificial Sequence
  Synthetic aptamer sequence
gggaagagaaggacatatgataaattgatctattcttttcggtgctatttatcttccatttttgactagtacatgaccactt

SEQ ID NO: 132 - DNA, 82 bp, Artificial Sequence
  Synthetic aptamer sequence
gggaagagaaggacatatgatctactcgcgcggcggacaaaagcgcaacccagcacccatgttgactagtacatgaccactt

SEQ ID NO: 133 - DNA, 82 bp, Artificial Sequence
  Synthetic aptamer sequence
gggaagagaaggacatatgattcttagtttgtaattacttttccttccttttattctatttttgactagtacatgaccactt

SEQ ID NO: 134 - DNA, 82 bp, Artificial Sequence
  Synthetic aptamer sequence
gggaagagaaggacatatgataacccgcgcagacttacaagcgcgcaaaaaaagggtacgtttgactagtacatgaccactt

SEQ ID NO: 135 - DNA, 82 bp, Artificial Sequence
  Synthetic aptamer sequence
gggaagagaaggacatatgatattcctttatgccgcatcattttattgtttatgacaatttttgactagtacatgaccactt

SEQ ID NO: 136 - DNA, 82 bp, Artificial Sequence
  Synthetic aptamer sequence
gggaagagaaggacatatgatatttcgtactacttttcttccaagcttcaatcgcccatttttgactagtacatgaccactt

SEQ ID NO: 137 - DNA, 82 bp, Artificial Sequence
  Synthetic aptamer sequence
gggaagagaaggacatatgattcactcattcgcaacacaattgtattcgcatctgcgatttttgactagtacatgaccactt

SEQ ID NO: 138 - DNA, 82 bp, Artificial Sequence
  Synthetic aptamer sequence
gggaagagaaggacatatgatattatttccacagttcctttatccacacatcttctcatttttgactagtacatgaccactt

SEQ ID NO: 139 - DNA, 82 bp, Artificial Sequence
  Synthetic aptamer sequence
gggaagagaaggacatatgataaactcgttatctattcgtttatttgcatctctttcatttttgactagtacatgaccactt

SEQ ID NO: 140 - DNA, 82 bp, Artificial Sequence
  Synthetic aptamer sequence
gggaagagaaggacatatgatccaacctctaaagtactggtcgcctagggagactgttcggttgactagtacatgaccactt

SEQ ID NO: 141 - DNA, 82 bp, Artificial Sequence
  Synthetic aptamer sequence
gggaagagaaggacatatgatttcctttttgctatttccgttaatgtaaactctcctatttttgactagtacatgaccactt

SEQ ID NO: 142 - DNA, 82 bp, Artificial Sequence
  Synthetic aptamer sequence
gggaagagaaggacatatgatccttatggcctagtagggatccgggcgccgaccagcgcgattgactagtacatgaccactt

SEQ ID NO: 143 - DNA, 82 bp, Artificial Sequence
  Synthetic aptamer sequence
gggaagagaaggacatatgatcgtctgtcttcttcgaatacgttttgggctaagcccatttttgactagtacatgaccactt

SEQ ID NO: 144 - DNA, 82 bp, Artificial Sequence
  Synthetic aptamer sequence
gggaagagaaggacatatgattcaaccaaactgccgacgaccgaggtatgtccttatgtacttgactagtacatgaccactt

SEQ ID NO: 145 - DNA, 82 bp, Artificial Sequence
  Synthetic aptamer sequence
gggaagagaaggacatatgattacgggtctgagcaaaagcgaaggaagcaggcgcagggatttgactagtacatgaccactt

SEQ ID NO: 146 - DNA, 82 bp, Artificial Sequence
  Synthetic aptamer sequence
gggaagagaaggacatatgattctctcattcgcaacacaattgtattcgcatctgcgatttttgactagtacatgaccactt

SEQ ID NO: 147 - DNA, 82 bp, Artificial Sequence
  Synthetic aptamer sequence
gggaagagaaggacatatgatgctctaaagtactaagcgtttgcgccgatgcccggaccgcttgactagtacatgaccactt

SEQ ID NO: 148 - DNA, 82 bp, Artificial Sequence
  Synthetic aptamer sequence
gggaagagaaggacatatgatacttcattaatgtgaggccgtcagggggcaaccttcgagcttgactagtacatgaccactt

SEQ ID NO: 149 - DNA, 82 bp, Artificial Sequence
  Synthetic aptamer sequence
gggaagagaaggacatatgattccttattcttgttactactttcttttcctatttttttctttgactagtacatgaccactt

SEQ ID NO: 150 - DNA, 82 bp, Artificial Sequence
  Synthetic aptamer sequence
gggaagagaaggacatatgatcgttattttcattttcttgttccccatatgcccaggcgcattgactagtacatgaccactt

SEQ ID NO: 151 - DNA, 82 bp, Artificial Sequence
  Synthetic aptamer sequence
gggaagagaaggacatatgataccagcggcgtagaaacgtacagctcgcctgtaacgcctgttgactagtacatgaccactt

SEQ ID NO: 152 - DNA, 82 bp, Artificial Sequence
  Synthetic aptamer sequence
gggaagagaaggacatatgatcgatatgggtgcgggaatgtacgttcaccgaatatgctccttgactagtacatgaccactt

SEQ ID NO: 153 - DNA, 82 bp, Artificial Sequence
  Synthetic aptamer sequence
gggaagagaaggacatatgattaacagtgcgtagtcatatcgaatgtttatcttcctatttttgactagtacatgaccactt

SEQ ID NO: 154 - DNA, 82 bp, Artificial Sequence
  Synthetic aptamer sequence
gggaagagaaggacatatgatcagactctcgcccaattcgcaaggcgttgcattgcgatttttgactagtacatgaccactt

SEQ ID NO: 155 - DNA, 82 bp, Artificial Sequence
  Synthetic aptamer sequence
gggaagagaaggacatatgatttccaactctccacgagagcatgggtcgaatgactcatttttgactagtacatgaccactt

SEQ ID NO: 156 - DNA, 82 bp, Artificial Sequence
  Synthetic aptamer sequence
gggaagagaaggacatatgatgcatcgcgcgtcactcaactcgtgattaccgagggcgccgttgactagtacatgaccactt

SEQ ID NO: 157 - DNA, 82 bp, Artificial Sequence
  Synthetic aptamer sequence
gggaagagaaggacatatgatctgaatctttccgcagccctgtccttttaaagacaggtttttgactagtacatgaccactt

SEQ ID NO: 158 - DNA, 82 bp, Artificial Sequence
  Synthetic aptamer sequence
gggaagagaaggacatatgattttgttacttacttcgtctatcttctgttgcacacagtttttgactagtacatgaccactt

SEQ ID NO: 159 - DNA, 82 bp, Artificial Sequence
  Synthetic aptamer sequence
gggaagagaaggacatatgattcaaatcttcagcgataatggcacaatttccgcgccatttttgactagtacatgaccactt

SEQ ID NO: 160 - DNA, 82 bp, Artificial Sequence
  Synthetic aptamer sequence
gggaagagaaggacatatgatttatgtgagatgatgtgtgttcctagttttatcttgctctttgactagtacatgaccactt

SEQ ID NO: 161 - DNA, 82 bp, Artificial Sequence
  Synthetic aptamer sequence
gggaagagaaggacatatgatccacttttccattaactgttgcgggcaagtagcaccgtttttgactagtacatgaccactt

SEQ ID NO: 162 - DNA, 82 bp, Artificial Sequence
  Synthetic aptamer sequence
gggaagagaaggacatatgatagagaagaccattcggaaagagctgcgtgtccttatgtacttgactagtacatgaccactt

SEQ ID NO: 163 - DNA, 82 bp, Artificial Sequence
  Synthetic aptamer sequence
gggaagagaaggacatatgattcttatgtagcaagcaaaatgtgccgccgagccgacgccattgactagtacatgaccactt

SEQ ID NO: 164 - DNA, 82 bp, Artificial Sequence
  Synthetic aptamer sequence
gggaagagaaggacatatgataagcgcataataagccagccagttcttggcgcgcggggtattgactagtacatgaccactt

SEQ ID NO: 165 - DNA, 82 bp, Artificial Sequence
  Synthetic aptamer sequence
gggaagagaaggacatatgattagtccgcatttctattttctatatggcttactgccatttttgactagtacatgaccactt

SEQ ID NO: 166 - DNA, 82 bp, Artificial Sequence
  Synthetic aptamer sequence
gggaagagaaggacatatgatataaagaacacgcaaaaccacccggacacccggtgccgtgttgactagtacatgaccactt

SEQ ID NO: 167 - DNA, 82 bp, Artificial Sequence
  Synthetic aptamer sequence
gggaagagaaggacatatgatacacaggcggtggagccgaagggcaccgggacaaaccgacttgactagtacatgaccactt

SEQ ID NO: 168 - DNA, 82 bp, Artificial Sequence
  Synthetic aptamer sequence
gggaagagaaggacatatgatagttccggcgcagcagcgtcctcacgttttacgtgccccattgactagtacatgaccactt

SEQ ID NO: 169 - DNA, 82 bp, Artificial Sequence
  Synthetic aptamer sequence
gggaagagaaggacatatgatgaccgtcgcgatcgtttataatgttctggatctttcatttttgactagtacatgaccactt

SEQ ID NO: 170 - DNA, 82 bp, Artificial Sequence
  Synthetic aptamer sequence
gggaagagaaggacatatgataagtggggccccgacgacttttccttcctctcttccggcattgactagtacatgaccactt

SEQ ID NO: 171 - DNA, 82 bp, Artificial Sequence
  Synthetic aptamer sequence
gggaagagaaggacatatgatatcaacataccaaaatgtcatttccaatcttttcccatttttgactagtacatgaccactt

SEQ ID NO: 172 - DNA, 82 bp, Artificial Sequence
  Synthetic aptamer sequence
gggaagagaaggacatatgatagcgaacaaacaagggtgcccaggcccccttcgcacatcgttgactagtacatgaccactt

SEQ ID NO: 173 - DNA, 82 bp, Artificial Sequence
  Synthetic aptamer sequence
gggaagagaaggacatatgatcctctgtaacgcaaagtcaagtcgcgcaaggccgcccgcgttgactagtacatgaccactt

SEQ ID NO: 174 - DNA, 82 bp, Artificial Sequence
  Synthetic aptamer sequence
gggaagagaaggacatatgatcttcatctgcgattacggtacactttagtgtatcgtttttttgactagtacatgaccactt

SEQ ID NO: 175 - DNA, 82 bp, Artificial Sequence
  Synthetic aptamer sequence
gggaagagaaggacatatgatgcctatgtgctagatgcagcagcaaccgccggcgactggattgactagtacatgaccactt

SEQ ID NO: 176 - DNA, 82 bp, Artificial Sequence
  Synthetic aptamer sequence
gggaagagaaggacatatgatccgcgccctaaccttctgaccaagcttccctggcacttggttgactagtacatgaccactt

SEQ ID NO: 177 - DNA, 82 bp, Artificial Sequence
  Synthetic aptamer sequence
gggaagagaaggacatatgatccttatgtattatcagtcataccggacgcagcccgctggattgactagtacatgaccactt

SEQ ID NO: 178 - DNA, 82 bp, Artificial Sequence
  Synthetic aptamer sequence
gggaagagaaggacatatgatctaatctatactggctgctaacgctttttcttttccatttttgactagtacatgaccactt

SEQ ID NO: 179 - DNA, 82 bp, Artificial Sequence
  Synthetic aptamer sequence
gggaagagaaggacatatgatcagtttacgcggagtcgtttgtgtccatttcttctcatttttgactagtacatgaccactt

SEQ ID NO: 180 - DNA, 82 bp, Artificial Sequence
  Synthetic aptamer sequence
gggaagagaaggacatatgattcacgtgagatgatgtgtgttcctagttttatcttgctctttgactagtacatgaccactt

SEQ ID NO: 181 - DNA, 82 bp, Artificial Sequence
  Synthetic aptamer sequence
gggaagagaaggacatatgattccttgtgtaccgctccgaatgtgctccagcgcgcctcggttgactagtacatgaccactt

SEQ ID NO: 182 - DNA, 82 bp, Artificial Sequence
  Synthetic aptamer sequence
gggaagagaaggacatatgataagccggcccgggaacatgtcacgcgcgcgcgcaaagtagttgactagtacatgaccactt

SEQ ID NO: 183 - DNA, 82 bp, Artificial Sequence
  Synthetic aptamer sequence
gggaagagaaggacatatgatcctggatttccgaaattagagtgccgtttcgttacggtttttgactagtacatgaccactt

SEQ ID NO: 184 - DNA, 82 bp, Artificial Sequence
  Synthetic aptamer sequence
gggaagagaaggacatatgatcgtgtcatccgcacaaggaggcctgcatggcagggacacgttgactagtacatgaccactt

SEQ ID NO: 185 - DNA, 82 bp, Artificial Sequence
  Synthetic aptamer sequence
gggaagagaaggacatatgatgagtagactttttgtatcatttttttatcgtaagatatttttgactagtacatgaccactt

SEQ ID NO: 186 - DNA, 82 bp, Artificial Sequence
  Synthetic aptamer sequence
gggaagagaaggacatatgatccatgtgagatgatgtgtgttcctagttttatcttgctctttgactagtacatgaccactt

SEQ ID NO: 187 - DNA, 82 bp, Artificial Sequence
  Synthetic aptamer sequence
gggaagagaaggacatatgatctttgctctagagtgtagtctatgagggacaaggtagccattgactagtacatgaccactt

SEQ ID NO: 188 - DNA, 82 bp, Artificial Sequence
  Synthetic aptamer sequence
gggaagagaaggacatatgatgttggttttctttctctttcttttctttctctttctatttttgactagtacatgaccactt

SEQ ID NO: 189 - DNA, 82 bp, Artificial Sequence
  Synthetic aptamer sequence
gggaagagaaggacatatgatcaatcgggcgggggtaagaggcgtgcgcagcgtggaggtgttgactagtacatgaccactt

SEQ ID NO: 190 - DNA, 82 bp, Artificial Sequence
  Synthetic aptamer sequence
gggaagagaaggacatatgatcaccgtggtgcgcaaagccgcaacgagaactgcggaatcgttgactagtacatgaccactt

SEQ ID NO: 191 - DNA, 82 bp, Artificial Sequence
  Synthetic aptamer sequence
gggaagagaaggacatatgattgctttaagtctttttatcattttgtttccttcattttttttgactagtacatgaccactt

SEQ ID NO: 192 - DNA, 82 bp, Artificial Sequence
  Synthetic aptamer sequence
gggaagagaaggacatatgatcgactagttatactgcaaaggctataagcgcgagcgcgcgttgactagtacatgaccactt

SEQ ID NO: 193 - DNA, 82 bp, Artificial Sequence
  Synthetic aptamer sequence
gggaagagaaggacatatgatgagtaatagatggcgtacacaaatcggatacgacgagcgcttgactagtacatgaccactt

SEQ ID NO: 194 - DNA, 82 bp, Artificial Sequence
  Synthetic aptamer sequence
gggaagagaaggacatatgattttcgcttcaagattcccaacgccttgtaagtcaaggtttttgactagtacatgaccactt

SEQ ID NO: 195 - DNA, 82 bp, Artificial Sequence
  Synthetic aptamer sequence
gggaagagaaggacatatgatgtgtgagatgagcccctggaccagacgcacgctcgcactgttgactagtacatgaccactt

SEQ ID NO: 196 - DNA, 82 bp, Artificial Sequence
  Synthetic aptamer sequence
gggaagagaaggacatatgatcaggatgcggcgccggtaattgacttccccctacgtaggattgactagtacatgaccactt

SEQ ID NO: 197 - DNA, 82 bp, Artificial Sequence
  Synthetic aptamer sequence
gggaagagaaggacatatgatcagggacccggccggtgcatctccttctttagcgtacgccttgactagtacatgaccactt

SEQ ID NO: 198 - DNA, 82 bp, Artificial Sequence
  Synthetic aptamer sequence
gggaagagaaggacatatgatctgctctaaagtaccaaccgcgggagctaaatgcaagccgttgactagtacatgaccactt

SEQ ID NO: 199 - DNA, 82 bp, Artificial Sequence
  Synthetic aptamer sequence
gggaagagaaggacatatgatgattgccatgcattagggggggacgcgcgcgaaagggagattgactagtacatgaccactt

SEQ ID NO: 200 - DNA, 82 bp, Artificial Sequence
  Synthetic aptamer sequence
gggaagagaaggacatatgattcgctctaaagtaccaaccgcgggagctaaatgcaagccgttgactagtacatgaccactt

SEQ ID NO: 201 - DNA, 82 bp, Artificial Sequence
  Synthetic aptamer sequence
gggaagagaaggacatatgataaaaaaccggggttcttaattttcattgttcgtcgtacttttgactagtacatgaccactt

SEQ ID NO: 202 - DNA, 82 bp, Artificial Sequence
  Synthetic aptamer sequence
gggaagagaaggacatatgataacccattggtgaatcgcaaccacagccagcccggcgcgattgactagtacatgaccactt

SEQ ID NO: 203 - DNA, 82 bp, Artificial Sequence
  Synthetic aptamer sequence
gggaagagaaggacatatgatcgaagtgaggggatcgcgcggggtgcacctaaatatgggattgactagtacatgaccactt

SEQ ID NO: 204 - DNA, 82 bp, Artificial Sequence
  Synthetic aptamer sequence
gggaagagaaggacatatgatagccttatgtactatagaagtcagctatccgccgcacaatttgactagtacatgaccactt

SEQ ID NO: 205 - DNA, 82 bp, Artificial Sequence
  Synthetic aptamer sequence
gggaagagaaggacatatgatcgttgtttttcccaaagctcgttagcattcattcctatttttgactagtacatgaccactt

SEQ ID NO: 206 - DNA, 82 bp, Artificial Sequence
  Synthetic aptamer sequence
gggaagagaaggacatatgatgatcatcagcggaaagcacgaaacgccacgggccgcggcattgactagtacatgaccactt

SEQ ID NO: 207 - DNA, 82 bp, Artificial Sequence
  Synthetic aptamer sequence
gggaagagaaggacatatgattccttcctattgacaatgcgcccgggcctcttcaattgtattgactagtacatgaccactt

SEQ ID NO: 208 - DNA, 82 bp, Artificial Sequence
  Synthetic aptamer sequence
gggaagagaaggacatatgatagttgccgcgcggcgcaagattggagagtcccgggctgtattgactagtacatgaccactt

SEQ ID NO: 209 - DNA, 82 bp, Artificial Sequence
  Synthetic aptamer sequence
gggaagagaaggacatatgatcataagttcgttcattccgttaacacgcgtatggcgttttttgactagtacatgaccactt

SEQ ID NO: 210 - DNA, 82 bp, Artificial Sequence
  Synthetic aptamer sequence
gggaagagaaggacatatgatcctttgtctccaaatcttaggactgaatgagtgcctatttttgactagtacatgaccactt

SEQ ID NO: 211 - DNA, 82 bp, Artificial Sequence
  Synthetic aptamer sequence
gggaagagaaggacatatgatcttctttgagaattctctttttacaattccggcgccgtgattgactagtacatgaccactt

SEQ ID NO: 212 - DNA, 82 bp, Artificial Sequence
  Synthetic aptamer sequence
gggaagagaaggacatatgattaggctaactgtttagggatttgatatgcatgaggagcacttgactagtacatgaccactt

SEQ ID NO: 213 - DNA, 82 bp, Artificial Sequence; identical to SEQ ID NO: 143
  Synthetic aptamer sequence

SEQ ID NO: 214 - DNA, 82 bp, Artificial Sequence
  Synthetic aptamer sequence
gggaagagaaggacatatgattaggctaactgctcagggatttgatatgcatgaggagcacttgactagtacatgaccactt

SEQ ID NO: 215 - DNA, 82 bp, Artificial Sequence
  Synthetic aptamer sequence
gggaagagaaggacatatgattaggctaactgttcagggacttgatatgcatgaggagcacttgactagtacatgaccactt

SEQ ID NO: 216 - DNA, 82 bp, Artificial Sequence
  Synthetic aptamer sequence
gggaagagaaggacatatgattaggctcactgttcagggatttgatatgcatgaggagcacttgactagtacatgaccactt

SEQ ID NO: 217 - DNA, 82 bp, Artificial Sequence
  Synthetic aptamer sequence
gggaagagaaggacatatgattaggctaactgttcagggatttgatatgcatggggagcacttgactagtacatgaccactt

SEQ ID NO: 218 - DNA, 82 bp, Artificial Sequence
  Synthetic aptamer sequence
gggaagagaaggacatatgatttcttcctattgacgatgcgcccgggcctcttcaattgtattgactagtacatgaccactt

SEQ ID NO: 219 - DNA, 82 bp, Artificial Sequence
  Synthetic aptamer sequence
gggaagagaaggacatatgattaggctaactgttcggggatttgatatgcatgaggagcacttgactagtacatgaccactt

SEQ ID NO: 220 - DNA, 82 bp, Artificial Sequence
  Synthetic aptamer sequence
gggaagagaaggacatatgattaggctaactgttcagggatttgatatgcacgaggagcacttgactagtacatgaccactt

SEQ ID NO: 221 - DNA, 82 bp, Artificial Sequence
  Synthetic aptamer sequence
gggaagagaaggacatatgattaggttaactgttcagggatttgatatgcatgaggagcacttgactagtacatgaccactt

SEQ ID NO: 222 - DNA, 82 bp, Artificial Sequence
  Synthetic aptamer sequence
gggaagagaaggacatatgattaggctaactgttcagggatttgatgtgcatgaggagcacttgactagtacatgaccactt